European Patent Application EP 4 219 698 A1, published August 2, 2023. Title: Peptide and use thereof in the prevention of therapy-related leukemia. Applicant: Universität Duisburg-Essen; Universität Ulm. The sequence listing filed with the application follows.

SEQUENCE LISTING (16 sequences)

SEQ ID NO: 1 - protein, 9 aa, Artificial
  Modified fragment of Ku80
  mics_feature (2)..(2): a linker which links the adjoining amino acids or an amino acid deletion
  mics_feature (5)..(5): a linker which links the adjoining amino acids or an amino acid deletion
EXEAXSGSS

SEQ ID NO: 2 - protein, 7 aa, Artificial
  Fragment of Ku80
EEASGSS

SEQ ID NO: 3 - protein, 28 aa, Artificial
  Fragment of Ku80
EIVVQDGITLITKEEASGSSVTAEEAKK

SEQ ID NO: 4 - protein, 21 aa, Artificial
  Fragment of Ku80
ITKEEASGSSVTAEEAKKFLA

SEQ ID NO: 5 - protein, 22 aa, Artificial
  Modified fragment of Ku80
ITKEEASGSSVTAEEAKKFLAG

SEQ ID NO: 6 - protein, 22 aa, Artificial
  Fragment of Ku80
ITKEEASGSSVTAEEAKKFLAP

SEQ ID NO: 7 - protein, 8 aa, Artificial
  Modified fragment of Ku80
  misc_feature (2)..(2): one or two amino acids selected from the group of glutamic acid, serine, alanine, and glycine
EXEASGSS

SEQ ID NO: 8 - protein, 28 aa, Artificial
  Scrambled peptide
VDSTTIEKSIAEVAEEQESILKKVAGGT

SEQ ID NO: 9 - protein, 26 aa, Artificial
  Fragment of Ku80
RVLVKQKKASFEEASNQLINHIEQFL

SEQ ID NO: 10 - protein, 30 aa, Artificial
  Fragment of Ku80
ASFEEASNQLINHIEQFLDTNETPYFMKSI

SEQ ID NO: 11 - DNA, 23 bp, Artificial
  primer
ttgggtgtaatcagttgcctatt

SEQ ID NO: 12 - DNA, 20 bp, Artificial
  primer
gggtgatagctgtttcggca

SEQ ID NO: 13 - DNA, 22 bp, Artificial
  primer
gcaacacagggccctagttaat

SEQ ID NO: 14 - DNA, 25 bp, Artificial
  primer
aggcaaatcagtcaccttttaatca

SEQ ID NO: 15 - protein, 7 aa, Artificial
  NLS motif of Ku80
PTAKKLK

SEQ ID NO: 16 - protein, 28 aa, Artificial
  Modified fragment of Ku80
EIVVQDGITLITKAEASGSSVTAEEAKK